European Patent Specification EP 3 054 766 B1, published June 18, 2025. Title: METHODS AND COMPOSITIONS FOR PERONOSPORA RESISTANCE IN SPINACH. Applicant: Seminis Vegetable Seeds, Inc. The sequence listing filed with the application follows.

SEQUENCE LISTING (4 sequences)

SEQ ID NO: 1 - DNA, 148 bp, Spinacia tetrandra
gcaaatagatgtgaaataactttttacatatgcaaatatattggaaatagcgaattatatatataatatggtttacataggtttcgacagagggcttactcgtatttatttgaataatatgtcatatttgacgagaataagaatgact

SEQ ID NO: 2 - DNA, 148 bp, Spinacia tetrandra
gctgctgcatcatagggtgatagttccttcctttttcctttatcattggtagatcgtttggcaaaagcctgtggcaccaatacaacaaaaggttaagataaatttgtttgctatgaccatattctaatcaaaagaacatagcaacata

SEQ ID NO: 3 - DNA, 120 bp, Spinacia oleracea
gcaaatagaagtgaaatagcgaatatatattatataatatggtttacatagatttcgacagaggggttactcgtatttgtttgaataatatttcatatttgatgaaaaatagggattact

SEQ ID NO: 4 - DNA, 150 bp, Spinacia oleracea
gctgctgcatcatagggtgatagttccttcctttttcctttatcattggtagatcttttggcaaaagcctgtatggcaccaatacaacaaaaggttaagataaatttgtttgctatgaccatattctaatcaaaagaacatagcaacata